European Patent Application EP 4 582 455 A1, published July 9, 2025. Title: 包含TACI多肽的融合蛋白及其用途. Applicant: 江苏恒瑞医药股份有限公司. Application WO. The sequence listing filed with the application follows.

SEQUENCE LISTING (78 sequences)

SEQ ID NO: 1 - protein, 165 aa, Homo sapiens
  source 1..165: note = TACI-ECD
MSGLGRSRRGGRSRVDQEERFPQGLWTGVAMRSCPEEQYWDPLLGTCMSCKTICNHQSQRTCAAFCRSLSCRKEQGKFYDHLLRDCISCASICGQHPKQCAYFCENKLRSPVNLPPELRRQRSGEVENNSDNSGRYQGLEHRGSEASPALPGLKLSADQVALVYS

SEQ ID NO: 2 - protein, 41 aa, synthetic construct
  source 1..41: note = TACI-9
SLSCRKEQGKFYDHLLRDCISCASICGQHPKQCAYFCENKL

SEQ ID NO: 3 - protein, 227 aa, Homo sapiens
  source 1..227: note; note (original language) = 人IgG1的Fc序列
DKTHTCPPCPAPEAEGAPSVFLFPPKPKDTLMISRTPEVTCVVVDVSHEDPEVKFNWYVDGVEVHNAKTKPREEQYNSTYRVVSVLTVLHQDWLNGKEYKCKVSNKALPSSIEKTISKAKGQPREPQVYTLPPSRDELTKNQVSLTCLVKGFYPSDIAVEWESNGQPENNYKTTPPVLDSDGSFFLYSKLTVDKSRWQQGNVFSCSVMHEALHNHYTQKSLSLSPGK

SEQ ID NO: 4 - protein, 333 aa, synthetic construct
  source 1..333: note = Telitacicept(RCT-18)
SRVDQEERFPQGLWTGVAMRSCPEEQYWDPLLGTCMSCKTICNHQSQRTCAAFCRSLSCRKEQGKFYDHLLRDCISCASICGQHPKQCAYFCENKLRSPVNLPPELDKTHTCPPCPAPEAEGAPSVFLFPPKPKDTLMISRTPEVTCVVVDVSHEDPEVKFNWYVDGVEVHNAKTKPREEQYNSTYRVVSVLTVLHQDWLNGKEYKCKVSNKALPSSIEKTISKAKGQPREPQVYTLPPSRDELTKNQVSLTCLVKGFYPSDIAVEWESNGQPENNYKTTPPVLDSDGSFFLYSKLTVDKSRWQQGNVFSCSVMHEALHNHYTQKSLSLSPGK

SEQ ID NO: 5 - protein, 313 aa, synthetic construct
  source 1..313: note = Atacicept
AMRSCPEEQYWDPLLGTCMSCKTICNHQSQRTCAAFCRSLSCRKEQGKFYDHLLRDCISCASICGQHPKQCAYFCENKLRSEPKSSDKTHTCPPCPAPEAEGAPSVFLFPPKPKDTLMISRTPEVTCVVVDVSHEDPEVKFNWYVDGVEVHNAKTKPREEQYNSTYRVVSVLTVLHQDWLNGKEYKCKVSNKALPSSIEKTISKAKGQPREPQVYTLPPSRDELTKNQVSLTCLVKGFYPSDIAVEWESNGQPENNYKTTPPVLDSDGSFFLYSKLTVDKSRWQQGNVFSCSVMHEALHNHYTQKSLSLSPGK

SEQ ID NO: 6 - protein, 40 aa, synthetic construct
  source 1..40: note = TACI-10
SLSCRKEQGKFYDHLLRDCISCASICGQHPKQCAYFCENK

SEQ ID NO: 7 - protein, 39 aa, synthetic construct
  source 1..39: note = TACI-11
SLSCRKEQGKFYDHLLRDCISCASICGQHPKQCAYFCEN

SEQ ID NO: 8 - protein, 38 aa, synthetic construct
  source 1..38: note = TACI-12
SLSCRKEQGKFYDHLLRDCISCASICGQHPKQCAYFCE

SEQ ID NO: 9 - protein, 41 aa, synthetic construct
  source 1..41: note = TACI-9-1
STSCRKEQGKFYDHLLRDCISCASICGQHPKQCAYFCENKL

SEQ ID NO: 10 - protein, 41 aa, synthetic construct
  source 1..41: note = TACI-9-2
SLSCSKEQGKFYDHLLRDCISCASICGQHPKQCAYFCENKL

SEQ ID NO: 11 - protein, 41 aa, synthetic construct
  source 1..41: note = TACI-9-3
SLSCREEQGKFYDHLLRDCISCASICGQHPKQCAYFCENKL

SEQ ID NO: 12 - protein, 41 aa, synthetic construct
  source 1..41: note = TACI-9-4
SLSCRQEQGKFYDHLLRDCISCASICGQHPKQCAYFCENKL

SEQ ID NO: 13 - protein, 41 aa, synthetic construct
  source 1..41: note = TACI-9-5
SLSCRKEQGEFYDHLLRDCISCASICGQHPKQCAYFCENKL

SEQ ID NO: 14 - protein, 41 aa, synthetic construct
  source 1..41: note = TACI-9-6
SRSCRKEQGKFYDHLLRTCISCASICGQHPKQCAYFCENKL

SEQ ID NO: 15 - protein, 41 aa, synthetic construct
  source 1..41: note = TACI-9-7
SRSCRKEQGKFYDHLLRACISCASICGQHPKQCAYFCENKL

SEQ ID NO: 16 - protein, 41 aa, synthetic construct
  source 1..41: note = TACI-9-8
SLSCRKEQGKFYDHLLRDCISCASICGQHPKQCAAFCENKL

SEQ ID NO: 17 - protein, 41 aa, synthetic construct
  source 1..41: note = TACI-9-9
SRSCRKEQGKFYDHLLRTCISCASICGQHPKQCARFCENKL

SEQ ID NO: 18 - protein, 41 aa, synthetic construct
  source 1..41: note = TACI-9-10
SLSCREEQGEFYDHLLRDCISCASICGQHPKQCAYFCENKL

SEQ ID NO: 19 - protein, 41 aa, synthetic construct
  source 1..41: note = TACI-9-11
SLSCSEEQGEFYDHLLRDCISCASICGQHPKQCAYFCENKL

SEQ ID NO: 20 - protein, 41 aa, synthetic construct
  source 1..41: note = TACI-9-12
STSCRKEQGKFYDHLLRDCISCASICGQHPKQCAAFCENKL

SEQ ID NO: 21 - protein, 41 aa, synthetic construct
  source 1..41: note = TACI-9-13
STSCRKEQGKFYDHLLRDCISCASICGQHPKQCAYYCENKL

SEQ ID NO: 22 - protein, 41 aa, synthetic construct
  source 1..41: note = TACI-9-14
STSCRKEQGKFYDHLLRDCISCASICGQHPKQCAAYCENKL

SEQ ID NO: 23 - protein, 41 aa, synthetic construct
  source 1..41: note = TACI-9-15
STSCREEQGEFYDHLLRDCISCASICGQHPKQCAAFCENKL

SEQ ID NO: 24 - protein, 40 aa, synthetic construct
  source 1..40: note = TACI-9-15a
STSCREEQGEFYDHLLRDCISCASICGQHPKQCAAFCENK

SEQ ID NO: 25 - protein, 39 aa, synthetic construct
  source 1..39: note = TACI-9-15b
STSCREEQGEFYDHLLRDCISCASICGQHPKQCAAFCEN

SEQ ID NO: 26 - protein, 38 aa, synthetic construct
  source 1..38: note = TACI-9-15c
STSCREEQGEFYDHLLRDCISCASICGQHPKQCAAFCE

SEQ ID NO: 27 - protein, 44 aa, synthetic construct
  source 1..44: note = TACI-d2
LSCRKEQGKFYDHLLRDCISCASICGQHPKQCAYFCENKLRSPG

SEQ ID NO: 28 - protein, 106 aa, synthetic construct
  source 1..106: note = TACI-T2
SRVDQEERFPQGLWTGVAMRSCPEEQYWDPLLGTCMSCKTICNHQSQRTCAAFCRSLSCRKEQGKFYDHLLRDCISCASICGQHPKQCAYFCENKLRSPVNLPPEL

SEQ ID NO: 29 - protein, 81 aa, synthetic construct
  source 1..81: note = TACI-T4
AMRSCPEEQYWDPLLGTCMSCKTICNHQSQRTCAAFCRSLSCRKEQGKFYDHLLRDCISCASICGQHPKQCAYFCENKLRS

SEQ ID NO: 30 - protein, 54 aa, synthetic construct
  source 1..54: note = BCMA-ECD
MLQMAGQCSQNEYFDSLLHACIPCQLRCSSNTPPLTCQRYCNASVTNSVKGTNA

SEQ ID NO: 31 - protein, 98 aa, synthetic construct
  source 1..98: note = TACI-d2-BCMA-ECD
LSCRKEQGKFYDHLLRDCISCASICGQHPKQCAYFCENKLRSPGMLQMAGQCSQNEYFDSLLHACIPCQLRCSSNTPPLTCQRYCNASVTNSVKGTNA

SEQ ID NO: 32 - protein, 98 aa, synthetic construct
  source 1..98: note = BCMA-ECD-TACI-d2
MLQMAGQCSQNEYFDSLLHACIPCQLRCSSNTPPLTCQRYCNASVTNSVKGTNALSCRKEQGKFYDHLLRDCISCASICGQHPKQCAYFCENKLRSPG

SEQ ID NO: 33 - protein, 160 aa, synthetic construct
  source 1..160: note = TACI-T2-BCMA-ECD
SRVDQEERFPQGLWTGVAMRSCPEEQYWDPLLGTCMSCKTICNHQSQRTCAAFCRSLSCRKEQGKFYDHLLRDCISCASICGQHPKQCAYFCENKLRSPVNLPPELMLQMAGQCSQNEYFDSLLHACIPCQLRCSSNTPPLTCQRYCNASVTNSVKGTNA

SEQ ID NO: 34 - protein, 160 aa, synthetic construct
  source 1..160: note = BCMA-ECD-TACI-T2
MLQMAGQCSQNEYFDSLLHACIPCQLRCSSNTPPLTCQRYCNASVTNSVKGTNASRVDQEERFPQGLWTGVAMRSCPEEQYWDPLLGTCMSCKTICNHQSQRTCAAFCRSLSCRKEQGKFYDHLLRDCISCASICGQHPKQCAYFCENKLRSPVNLPPEL

SEQ ID NO: 35 - protein, 325 aa, synthetic construct
  source 1..325: note = B575701
LSCRKEQGKFYDHLLRDCISCASICGQHPKQCAYFCENKLRSPGMLQMAGQCSQNEYFDSLLHACIPCQLRCSSNTPPLTCQRYCNASVTNSVKGTNADKTHTCPPCPAPEAEGAPSVFLFPPKPKDTLMISRTPEVTCVVVDVSHEDPEVKFNWYVDGVEVHNAKTKPREEQYNSTYRVVSVLTVLHQDWLNGKEYKCKVSNKALPSSIEKTISKAKGQPREPQVYTLPPSRDELTKNQVSLTCLVKGFYPSDIAVEWESNGQPENNYKTTPPVLDSDGSFFLYSKLTVDKSRWQQGNVFSCSVMHEALHNHYTQKSLSLSPGK

SEQ ID NO: 36 - protein, 325 aa, synthetic construct
  source 1..325: note = B575702
MLQMAGQCSQNEYFDSLLHACIPCQLRCSSNTPPLTCQRYCNASVTNSVKGTNALSCRKEQGKFYDHLLRDCISCASICGQHPKQCAYFCENKLRSPGDKTHTCPPCPAPEAEGAPSVFLFPPKPKDTLMISRTPEVTCVVVDVSHEDPEVKFNWYVDGVEVHNAKTKPREEQYNSTYRVVSVLTVLHQDWLNGKEYKCKVSNKALPSSIEKTISKAKGQPREPQVYTLPPSRDELTKNQVSLTCLVKGFYPSDIAVEWESNGQPENNYKTTPPVLDSDGSFFLYSKLTVDKSRWQQGNVFSCSVMHEALHNHYTQKSLSLSPGK

SEQ ID NO: 37 - protein, 387 aa, synthetic construct
  source 1..387: note = B575703
SRVDQEERFPQGLWTGVAMRSCPEEQYWDPLLGTCMSCKTICNHQSQRTCAAFCRSLSCRKEQGKFYDHLLRDCISCASICGQHPKQCAYFCENKLRSPVNLPPELMLQMAGQCSQNEYFDSLLHACIPCQLRCSSNTPPLTCQRYCNASVTNSVKGTNADKTHTCPPCPAPEAEGAPSVFLFPPKPKDTLMISRTPEVTCVVVDVSHEDPEVKFNWYVDGVEVHNAKTKPREEQYNSTYRVVSVLTVLHQDWLNGKEYKCKVSNKALPSSIEKTISKAKGQPREPQVYTLPPSRDELTKNQVSLTCLVKGFYPSDIAVEWESNGQPENNYKTTPPVLDSDGSFFLYSKLTVDKSRWQQGNVFSCSVMHEALHNHYTQKSLSLSPGK

SEQ ID NO: 38 - protein, 387 aa, synthetic construct
  source 1..387: note = B575704
MLQMAGQCSQNEYFDSLLHACIPCQLRCSSNTPPLTCQRYCNASVTNSVKGTNASRVDQEERFPQGLWTGVAMRSCPEEQYWDPLLGTCMSCKTICNHQSQRTCAAFCRSLSCRKEQGKFYDHLLRDCISCASICGQHPKQCAYFCENKLRSPVNLPPELDKTHTCPPCPAPEAEGAPSVFLFPPKPKDTLMISRTPEVTCVVVDVSHEDPEVKFNWYVDGVEVHNAKTKPREEQYNSTYRVVSVLTVLHQDWLNGKEYKCKVSNKALPSSIEKTISKAKGQPREPQVYTLPPSRDELTKNQVSLTCLVKGFYPSDIAVEWESNGQPENNYKTTPPVLDSDGSFFLYSKLTVDKSRWQQGNVFSCSVMHEALHNHYTQKSLSLSPGK

SEQ ID NO: 39 - protein, 10 aa, synthetic construct
  source 1..10: note; note (original language) = 连接子1
GGGGSGGGGS

SEQ ID NO: 40 - protein, 15 aa, synthetic construct
  source 1..15: note; note (original language) = 连接子2
GGGGSGGGGSGGGGS

SEQ ID NO: 41 - protein, 20 aa, synthetic construct
  source 1..20: note; note (original language) = 连接子3
GGGGSGGGGSGGGGSGGGGS

SEQ ID NO: 42 - protein, 38 aa, synthetic construct; identical to SEQ ID NO: 8
  source 1..38: note = TACI-CRD2

SEQ ID NO: 43 - protein, 117 aa, synthetic construct [sequence omitted]

SEQ ID NO: 44 - protein, 108 aa, synthetic construct [sequence omitted]

SEQ ID NO: 45 - protein, 5 aa, synthetic construct
  source 1..5: note = Anifrolumab HCDR1
NYWIA

SEQ ID NO: 46 - protein, 17 aa, synthetic construct
  source 1..17: note = Anifrolumab HCDR2
IIYPGDSDIRYSPSFQG

SEQ ID NO: 47 - protein, 8 aa, synthetic construct
  source 1..8: note = Anifrolumab HCDR3
HDIEGFDY

SEQ ID NO: 48 - protein, 12 aa, synthetic construct
  source 1..12: note = Anifrolumab LCDR1
RASQSVSSSFFA

SEQ ID NO: 49 - protein, 7 aa, synthetic construct
  source 1..7: note = Anifrolumab LCDR2
GASSRAT

SEQ ID NO: 50 - protein, 9 aa, synthetic construct
  source 1..9: note = Anifrolumab LCDR3
QQYDSSAIT

SEQ ID NO: 51 - protein, 538 aa, synthetic construct
  source 1..538: note; note (original language) = B385801的重链
AMRSCPEEQYWDPLLGTCMSCKTICNHQSQRTCAAFCRSLSCRKEQGKFYDHLLRDCISCASICGQHPKQCAYFCENKLRSGGGGSGGGGSEVQLVQSGAEVKKPGESLKISCKGSGYIFTNYWIAWVRQMPGKGLESMGIIYPGDSDIRYSPSFQGQVTISADKSITTAYLQWSSLKASDTAMYYCARHDIEGFDYWGRGTLVTVSSASTKGPSVFPLAPSSKSTSGGTAALGCLVKDYFPEPVTVSWNSGALTSGVHTFPAVLQSSGLYSLSSVVTVPSSSLGTQTYICNVNHKPSNTKVDKRVEPKSCDKTHTCPPCPAPEFEGGPSVFLFPPKPKDTLMISRTPEVTCVVVDVSHEDPEVKFNWYVDGVEVHNAKTKPREEQYNSTYRVVSVLTVLHQDWLNGKEYKCKVSNKALPASIEKTISKAKGQPREPQVYTLPPSRDELTKNQVSLTCLVKGFYPSDIAVEWESNGQPENNYKTTPPVLDSDGSFFLYSKLTVDKSRWQQGNVFSCSVMHEALHNHYTQKSLSLSPGK

SEQ ID NO: 52 - protein, 538 aa, synthetic construct
  source 1..538: note; note (original language) = B385802的重链
EVQLVQSGAEVKKPGESLKISCKGSGYIFTNYWIAWVRQMPGKGLESMGIIYPGDSDIRYSPSFQGQVTISADKSITTAYLQWSSLKASDTAMYYCARHDIEGFDYWGRGTLVTVSSASTKGPSVFPLAPSSKSTSGGTAALGCLVKDYFPEPVTVSWNSGALTSGVHTFPAVLQSSGLYSLSSVVTVPSSSLGTQTYICNVNHKPSNTKVDKRVEPKSCDKTHTCPPCPAPEFEGGPSVFLFPPKPKDTLMISRTPEVTCVVVDVSHEDPEVKFNWYVDGVEVHNAKTKPREEQYNSTYRVVSVLTVLHQDWLNGKEYKCKVSNKALPASIEKTISKAKGQPREPQVYTLPPSRDELTKNQVSLTCLVKGFYPSDIAVEWESNGQPENNYKTTPPVLDSDGSFFLYSKLTVDKSRWQQGNVFSCSVMHEALHNHYTQKSLSLSPGKGGGGSGGGGSAMRSCPEEQYWDPLLGTCMSCKTICNHQSQRTCAAFCRSLSCRKEQGKFYDHLLRDCISCASICGQHPKQCAYFCENKLRS

SEQ ID NO: 53 - protein, 500 aa, synthetic construct
  source 1..500: note; note (original language) = B805201的重链
EVQLVQSGAEVKKPGESLKISCKGSGYIFTNYWIAWVRQMPGKGLESMGIIYPGDSDIRYSPSFQGQVTISADKSITTAYLQWSSLKASDTAMYYCARHDIEGFDYWGRGTLVTVSSASTKGPSVFPLAPSSKSTSGGTAALGCLVKDYFPEPVTVSWNSGALTSGVHTFPAVLQSSGLYSLSSVVTVPSSSLGTQTYICNVNHKPSNTKVDKRVEPKSCDKTHTCPPCPAPEFEGGPSVFLFPPKPKDTLMISRTPEVTCVVVDVSHEDPEVKFNWYVDGVEVHNAKTKPREEQYNSTYRVVSVLTVLHQDWLNGKEYKCKVSNKALPASIEKTISKAKGQPREPQVYTLPPSRDELTKNQVSLTCLVKGFYPSDIAVEWESNGQPENNYKTTPPVLDSDGSFFLYSKLTVDKSRWQQGNVFSCSVMHEALHNHYTQKSLSLSPGKGGGGSGGGGSGGGGSSTSCREEQGEFYDHLLRDCISCASICGQHPKQCAAFCE

SEQ ID NO: 54 - protein, 215 aa, synthetic construct
  source 1..215: note; note (original language) = B385801、B385802、B805201、B805201-LALA的轻链
EIVLTQSPGTLSLSPGERATLSCRASQSVSSSFFAWYQQKPGQAPRLLIYGASSRATGIPDRLSGSGSGTDFTLTITRLEPEDFAVYYCQQYDSSAITFGQGTRLEIKRTVAAPSVFIFPPSDEQLKSGTASVVCLLNNFYPREAKVQWKVDNALQSGNSQESVTEQDSKDSTYSLSSTLTLSKADYEKHKVYACEVTHQGLSSPVTKSFNRGEC

SEQ ID NO: 55 - protein, 447 aa, synthetic construct
  source 1..447: note; note (original language) = B385803、B385804、B498301、B498302、B606401的重链
EVQLVQSGAEVKKPGESLKISCKGSGYIFTNYWIAWVRQMPGKGLESMGIIYPGDSDIRYSPSFQGQVTISADKSITTAYLQWSSLKASDTAMYYCARHDIEGFDYWGRGTLVTVSSASTKGPSVFPLAPSSKSTSGGTAALGCLVKDYFPEPVTVSWNSGALTSGVHTFPAVLQSSGLYSLSSVVTVPSSSLGTQTYICNVNHKPSNTKVDKRVEPKSCDKTHTCPPCPAPEFEGGPSVFLFPPKPKDTLMISRTPEVTCVVVDVSHEDPEVKFNWYVDGVEVHNAKTKPREEQYNSTYRVVSVLTVLHQDWLNGKEYKCKVSNKALPASIEKTISKAKGQPREPQVYTLPPSRDELTKNQVSLTCLVKGFYPSDIAVEWESNGQPENNYKTTPPVLDSDGSFFLYSKLTVDKSRWQQGNVFSCSVMHEALHNHYTQKSLSLSPGK

SEQ ID NO: 56 - protein, 306 aa, synthetic construct
  source 1..306: note; note (original language) = B385803的轻链
AMRSCPEEQYWDPLLGTCMSCKTICNHQSQRTCAAFCRSLSCRKEQGKFYDHLLRDCISCASICGQHPKQCAYFCENKLRSGGGGSGGGGSEIVLTQSPGTLSLSPGERATLSCRASQSVSSSFFAWYQQKPGQAPRLLIYGASSRATGIPDRLSGSGSGTDFTLTITRLEPEDFAVYYCQQYDSSAITFGQGTRLEIKRTVAAPSVFIFPPSDEQLKSGTASVVCLLNNFYPREAKVQWKVDNALQSGNSQESVTEQDSKDSTYSLSSTLTLSKADYEKHKVYACEVTHQGLSSPVTKSFNRGEC

SEQ ID NO: 57 - protein, 306 aa, synthetic construct
  source 1..306: note; note (original language) = B385804的轻链
EIVLTQSPGTLSLSPGERATLSCRASQSVSSSFFAWYQQKPGQAPRLLIYGASSRATGIPDRLSGSGSGTDFTLTITRLEPEDFAVYYCQQYDSSAITFGQGTRLEIKRTVAAPSVFIFPPSDEQLKSGTASVVCLLNNFYPREAKVQWKVDNALQSGNSQESVTEQDSKDSTYSLSSTLTLSKADYEKHKVYACEVTHQGLSSPVTKSFNRGECGGGGSGGGGSAMRSCPEEQYWDPLLGTCMSCKTICNHQSQRTCAAFCRSLSCRKEQGKFYDHLLRDCISCASICGQHPKQCAYFCENKLRS

SEQ ID NO: 58 - protein, 311 aa, synthetic construct
  source 1..311: note; note (original language) = B498301的轻链
EIVLTQSPGTLSLSPGERATLSCRASQSVSSSFFAWYQQKPGQAPRLLIYGASSRATGIPDRLSGSGSGTDFTLTITRLEPEDFAVYYCQQYDSSAITFGQGTRLEIKRTVAAPSVFIFPPSDEQLKSGTASVVCLLNNFYPREAKVQWKVDNALQSGNSQESVTEQDSKDSTYSLSSTLTLSKADYEKHKVYACEVTHQGLSSPVTKSFNRGECGGGGSGGGGSGGGGSAMRSCPEEQYWDPLLGTCMSCKTICNHQSQRTCAAFCRSLSCRKEQGKFYDHLLRDCISCASICGQHPKQCAYFCENKLRS

SEQ ID NO: 59 - protein, 316 aa, synthetic construct
  source 1..316: note; note (original language) = B498302的轻链
EIVLTQSPGTLSLSPGERATLSCRASQSVSSSFFAWYQQKPGQAPRLLIYGASSRATGIPDRLSGSGSGTDFTLTITRLEPEDFAVYYCQQYDSSAITFGQGTRLEIKRTVAAPSVFIFPPSDEQLKSGTASVVCLLNNFYPREAKVQWKVDNALQSGNSQESVTEQDSKDSTYSLSSTLTLSKADYEKHKVYACEVTHQGLSSPVTKSFNRGECGGGGSGGGGSGGGGSGGGGSAMRSCPEEQYWDPLLGTCMSCKTICNHQSQRTCAAFCRSLSCRKEQGKFYDHLLRDCISCASICGQHPKQCAYFCENKLRS

SEQ ID NO: 60 - protein, 263 aa, synthetic construct
  source 1..263: note; note (original language) = B606401、B606401-LALA的轻链
EIVLTQSPGTLSLSPGERATLSCRASQSVSSSFFAWYQQKPGQAPRLLIYGASSRATGIPDRLSGSGSGTDFTLTITRLEPEDFAVYYCQQYDSSAITFGQGTRLEIKRTVAAPSVFIFPPSDEQLKSGTASVVCLLNNFYPREAKVQWKVDNALQSGNSQESVTEQDSKDSTYSLSSTLTLSKADYEKHKVYACEVTHQGLSSPVTKSFNRGECGGGGSGGGGSSTSCREEQGEFYDHLLRDCISCASICGQHPKQCAAFCE

SEQ ID NO: 61 - protein, 447 aa, synthetic construct
  source 1..447: note; note (original language) = B606401-LALA的重链
EVQLVQSGAEVKKPGESLKISCKGSGYIFTNYWIAWVRQMPGKGLESMGIIYPGDSDIRYSPSFQGQVTISADKSITTAYLQWSSLKASDTAMYYCARHDIEGFDYWGRGTLVTVSSASTKGPSVFPLAPSSKSTSGGTAALGCLVKDYFPEPVTVSWNSGALTSGVHTFPAVLQSSGLYSLSSVVTVPSSSLGTQTYICNVNHKPSNTKVDKRVEPKSCDKTHTCPPCPAPEAAGGPSVFLFPPKPKDTLMISRTPEVTCVVVDVSHEDPEVKFNWYVDGVEVHNAKTKPREEQYNSTYRVVSVLTVLHQDWLNGKEYKCKVSNKALPAPIEKTISKAKGQPREPQVYTLPPSRDELTKNQVSLTCLVKGFYPSDIAVEWESNGQPENNYKTTPPVLDSDGSFFLYSKLTVDKSRWQQGNVFSCSVMHEALHNHYTQKSLSLSPGK

SEQ ID NO: 62 - protein, 500 aa, synthetic construct
  source 1..500: note; note (original language) = B805201-LALA的重链
EVQLVQSGAEVKKPGESLKISCKGSGYIFTNYWIAWVRQMPGKGLESMGIIYPGDSDIRYSPSFQGQVTISADKSITTAYLQWSSLKASDTAMYYCARHDIEGFDYWGRGTLVTVSSASTKGPSVFPLAPSSKSTSGGTAALGCLVKDYFPEPVTVSWNSGALTSGVHTFPAVLQSSGLYSLSSVVTVPSSSLGTQTYICNVNHKPSNTKVDKRVEPKSCDKTHTCPPCPAPEAAGGPSVFLFPPKPKDTLMISRTPEVTCVVVDVSHEDPEVKFNWYVDGVEVHNAKTKPREEQYNSTYRVVSVLTVLHQDWLNGKEYKCKVSNKALPAPIEKTISKAKGQPREPQVYTLPPSRDELTKNQVSLTCLVKGFYPSDIAVEWESNGQPENNYKTTPPVLDSDGSFFLYSKLTVDKSRWQQGNVFSCSVMHEALHNHYTQKSLSLSPGKGGGGSGGGGSGGGGSSTSCREEQGEFYDHLLRDCISCASICGQHPKQCAAFCE

SEQ ID NO: 63 - protein, 323 aa, synthetic construct
  source 1..323: note; note (original language) = B613301的轻链
EIVLTQSPGTLSLSPGERATLSCRASQSVSSSFFAWYQQKPGQAPRLLIYGASSRATGIPDRLSGSGSGTDFTLTITRLEPEDFAVYYCQQYDSSAITFGQGTRLEIKRTVAAPSVFIFPPSDEQLKSGTASVVCLLNNFYPREAKVQWKVDNALQSGNSQESVTEQDSKDSTYSLSSTLTLSKADYEKHKVYACEVTHQGLSSPVTKSFNRGECGGGGSGGGGSLSCRKEQGKFYDHLLRDCISCASICGQHPKQCAYFCENKLRSPGMLQMAGQCSQNEYFDSLLHACIPCQLRCSSNTPPLTCQRYCNASVTNSVKGTNA

SEQ ID NO: 64 - protein, 323 aa, synthetic construct
  source 1..323: note; note (original language) = B613302的轻链
EIVLTQSPGTLSLSPGERATLSCRASQSVSSSFFAWYQQKPGQAPRLLIYGASSRATGIPDRLSGSGSGTDFTLTITRLEPEDFAVYYCQQYDSSAITFGQGTRLEIKRTVAAPSVFIFPPSDEQLKSGTASVVCLLNNFYPREAKVQWKVDNALQSGNSQESVTEQDSKDSTYSLSSTLTLSKADYEKHKVYACEVTHQGLSSPVTKSFNRGECGGGGSGGGGSMLQMAGQCSQNEYFDSLLHACIPCQLRCSSNTPPLTCQRYCNASVTNSVKGTNALSCRKEQGKFYDHLLRDCISCASICGQHPKQCAYFCENKLRSPG

SEQ ID NO: 65 - protein, 385 aa, synthetic construct
  source 1..385: note; note (original language) = B613303的轻链
EIVLTQSPGTLSLSPGERATLSCRASQSVSSSFFAWYQQKPGQAPRLLIYGASSRATGIPDRLSGSGSGTDFTLTITRLEPEDFAVYYCQQYDSSAITFGQGTRLEIKRTVAAPSVFIFPPSDEQLKSGTASVVCLLNNFYPREAKVQWKVDNALQSGNSQESVTEQDSKDSTYSLSSTLTLSKADYEKHKVYACEVTHQGLSSPVTKSFNRGECGGGGSGGGGSSRVDQEERFPQGLWTGVAMRSCPEEQYWDPLLGTCMSCKTICNHQSQRTCAAFCRSLSCRKEQGKFYDHLLRDCISCASICGQHPKQCAYFCENKLRSPVNLPPELMLQMAGQCSQNEYFDSLLHACIPCQLRCSSNTPPLTCQRYCNASVTNSVKGTNA

SEQ ID NO: 66 - protein, 385 aa, synthetic construct
  source 1..385: note; note (original language) = B613304的轻链
EIVLTQSPGTLSLSPGERATLSCRASQSVSSSFFAWYQQKPGQAPRLLIYGASSRATGIPDRLSGSGSGTDFTLTITRLEPEDFAVYYCQQYDSSAITFGQGTRLEIKRTVAAPSVFIFPPSDEQLKSGTASVVCLLNNFYPREAKVQWKVDNALQSGNSQESVTEQDSKDSTYSLSSTLTLSKADYEKHKVYACEVTHQGLSSPVTKSFNRGECGGGGSGGGGSMLQMAGQCSQNEYFDSLLHACIPCQLRCSSNTPPLTCQRYCNASVTNSVKGTNASRVDQEERFPQGLWTGVAMRSCPEEQYWDPLLGTCMSCKTICNHQSQRTCAAFCRSLSCRKEQGKFYDHLLRDCISCASICGQHPKQCAYFCENKLRSPVNLPPEL

SEQ ID NO: 67 - protein, 43 aa, synthetic construct
  source 1..43: note = BCMA-ECD-1
MLQMAGQCSQNEYFDSLLHACIPCQLRCSSNTPPLTCQRYCNA

SEQ ID NO: 68 - protein, 41 aa, synthetic construct
  source 1..41: note = BCMA-ECD-2
MLQMAGQCSQNEYFDSLLHACIPCQLRCSSNTPPLTCQRYC

SEQ ID NO: 69 - protein, 81 aa, synthetic construct
  source 1..81: note = TACI-19-16-BCMA-ECD-1
STSCREEQGEFYDHLLRDCISCASICGQHPKQCAAFCEMLQMAGQCSQNEYFDSLLHACIPCQLRCSSNTPPLTCQRYCNA

SEQ ID NO: 70 - protein, 79 aa, synthetic construct
  source 1..79: note = BCMA-ECD-2-TACI-19-16
MLQMAGQCSQNEYFDSLLHACIPCQLRCSSNTPPLTCQRYCSTSCREEQGEFYDHLLRDCISCASICGQHPKQCAAFCE

SEQ ID NO: 71 - protein, 306 aa, synthetic construct
  source 1..306: note; note (original language) = B637301的轻链
EIVLTQSPGTLSLSPGERATLSCRASQSVSSSFFAWYQQKPGQAPRLLIYGASSRATGIPDRLSGSGSGTDFTLTITRLEPEDFAVYYCQQYDSSAITFGQGTRLEIKRTVAAPSVFIFPPSDEQLKSGTASVVCLLNNFYPREAKVQWKVDNALQSGNSQESVTEQDSKDSTYSLSSTLTLSKADYEKHKVYACEVTHQGLSSPVTKSFNRGECGGGGSGGGGSSTSCREEQGEFYDHLLRDCISCASICGQHPKQCAAFCEMLQMAGQCSQNEYFDSLLHACIPCQLRCSSNTPPLTCQRYCNA

SEQ ID NO: 72 - protein, 304 aa, synthetic construct
  source 1..304: note; note (original language) = B637302、B637302-LALA的轻链
EIVLTQSPGTLSLSPGERATLSCRASQSVSSSFFAWYQQKPGQAPRLLIYGASSRATGIPDRLSGSGSGTDFTLTITRLEPEDFAVYYCQQYDSSAITFGQGTRLEIKRTVAAPSVFIFPPSDEQLKSGTASVVCLLNNFYPREAKVQWKVDNALQSGNSQESVTEQDSKDSTYSLSSTLTLSKADYEKHKVYACEVTHQGLSSPVTKSFNRGECGGGGSGGGGSMLQMAGQCSQNEYFDSLLHACIPCQLRCSSNTPPLTCQRYCSTSCREEQGEFYDHLLRDCISCASICGQHPKQCAAFCE

SEQ ID NO: 73 - protein, 541 aa, synthetic construct
  source 1..541: note; note (original language) = B746201的重链
EVQLVQSGAEVKKPGESLKISCKGSGYIFTNYWIAWVRQMPGKGLESMGIIYPGDSDIRYSPSFQGQVTISADKSITTAYLQWSSLKASDTAMYYCARHDIEGFDYWGRGTLVTVSSASTKGPSVFPLAPSSKSTSGGTAALGCLVKDYFPEPVTVSWNSGALTSGVHTFPAVLQSSGLYSLSSVVTVPSSSLGTQTYICNVNHKPSNTKVDKRVEPKSCDKTHTCPPCPAPEFEGGPSVFLFPPKPKDTLMISRTPEVTCVVVDVSHEDPEVKFNWYVDGVEVHNAKTKPREEQYNSTYRVVSVLTVLHQDWLNGKEYKCKVSNKALPASIEKTISKAKGQPREPQVYTLPPSRDELTKNQVSLTCLVKGFYPSDIAVEWESNGQPENNYKTTPPVLDSDGSFFLYSKLTVDKSRWQQGNVFSCSVMHEALHNHYTQKSLSLSPGKGGGGSGGGGSGGGGSMLQMAGQCSQNEYFDSLLHACIPCQLRCSSNTPPLTCQRYCSTSCREEQGEFYDHLLRDCISCASICGQHPKQCAAFCE

SEQ ID NO: 74 - protein, 541 aa, synthetic construct
  source 1..541: note; note (original language) = B746201-LALA的重链
EVQLVQSGAEVKKPGESLKISCKGSGYIFTNYWIAWVRQMPGKGLESMGIIYPGDSDIRYSPSFQGQVTISADKSITTAYLQWSSLKASDTAMYYCARHDIEGFDYWGRGTLVTVSSASTKGPSVFPLAPSSKSTSGGTAALGCLVKDYFPEPVTVSWNSGALTSGVHTFPAVLQSSGLYSLSSVVTVPSSSLGTQTYICNVNHKPSNTKVDKRVEPKSCDKTHTCPPCPAPEAAGGPSVFLFPPKPKDTLMISRTPEVTCVVVDVSHEDPEVKFNWYVDGVEVHNAKTKPREEQYNSTYRVVSVLTVLHQDWLNGKEYKCKVSNKALPAPIEKTISKAKGQPREPQVYTLPPSRDELTKNQVSLTCLVKGFYPSDIAVEWESNGQPENNYKTTPPVLDSDGSFFLYSKLTVDKSRWQQGNVFSCSVMHEALHNHYTQKSLSLSPGKGGGGSGGGGSGGGGSMLQMAGQCSQNEYFDSLLHACIPCQLRCSSNTPPLTCQRYCSTSCREEQGEFYDHLLRDCISCASICGQHPKQCAAFCE

SEQ ID NO: 75 - protein, 5 aa, synthetic construct
  source 1..5: note; note (original language) = 连接子
  REGION 1..5: note = the entire sequence could be repeated 1-20 times.
GGNGT

SEQ ID NO: 76 - protein, 5 aa, synthetic construct
  source 1..5: note; note (original language) = 连接子
  REGION 1..5: note = the entire sequence could be repeated 1-20 times.
YGNGT

SEQ ID NO: 77 - protein, 5 aa, synthetic construct
  source 1..5: note; note (original language) = 连接子
  REGION 1..5: note = the entire sequence could be repeated 1-20 times.
EPKSS

SEQ ID NO: 78 - protein, 5 aa, synthetic construct
  source 1..5: note; note (original language) = 连接子
  REGION 1..5: note = the entire sequence could be repeated 1-6 times.
GGGGS